European Patent Specification EP 4 291 251 B1, published February 19, 2025. Title: NEW POLYPEPTIDE. Applicant: AFFIBODY AB. The sequence listing filed with the application follows.

SEQUENCE LISTING (6 sequences)

SEQ ID NO: 1 - protein, 59 aa, Artificial sequence
  Engineered HER2 binding polypeptide
AEAKYAKEMRNAYWEIALLPNLTNQQKRAFIRKLYDDPSQSSELLSEAKKLSESQGGGC

SEQ ID NO: 2 - protein, 59 aa, Artificial sequence
  Engineered HER2 binding polypeptide
AENKFNKEMRNAYWEIALLPNLTNQQKRAFIRSLYDDPSQSANLLAEAKKLNDAQGGGC

SEQ ID NO: 3 - protein, 61 aa, Artificial sequence
  Engineered HER2 binding polypeptide
AENKFNKEMRNAYWEIALLPNLTNQQKRAFIRSLYDDPSQSANLLAEAKKLNDAQAPKVDC

SEQ ID NO: 4 - protein, 4 aa, Artificial sequence
  C-terminal sequence in engineered polypeptide of e.g. Ahlgren et al 2009
KVDC

SEQ ID NO: 5 - protein, 4 aa, Artificial sequence
  C-terminal sequence in engineered polypeptide of the disclosure
GGGC

SEQ ID NO: 6 - protein, 6 aa, Artificial sequence
  N-terminal sequence in engineered polypeptide of e.g. Lindberg et al 2012
HEHEHE